European Patent Application EP 4 772 624 A1, published July 8, 2026. Title: IdeZ variant. Applicant: Astellas Pharma Inc. The sequence listing filed with the application follows.

SEQUENCE LISTING (35 sequences)

SEQ ID NO: 1 - protein, 349 aa, Streptococcus equi
MKTIAYPNKPHSLSAGLLTAIAIFSLASSNITYADDYQRNAAEVYAKEVPHQITSVWTKGVTPLTPEQFRYNNEDVIHAPYLAHQGWYDITKVFDGKDNLLCGAATAGNMLHWWFDQNKTEIEAYLSKHPEKQKIIFNNQELFDLKAAIDTKDSQTNSQLFNYFRDKAFPNLSARQLGVMPDLVLDMFINGYYLNVFKTQSTDVNRPYQDKDKRGGIFDAVFTRGDQTTLLTARHDLKNKGLNDISTIIKQELTEGRALALSHTYANVSISHVINLWGADFNAEGNLEAIYVTDSDANASIGMKKYFVGINAHGHVAISAKKIEGENIGAQVLGLFTLSSGKDIWQKLS

SEQ ID NO: 2 - DNA, 945 bp, Streptococcus equi
  source 1..945: mol_type = other DNA
gacgactaccagagaaacgccgccgaggtgtacgccaaagaggtgccacatcagatcacctccgtgtggaccaagggcgtgacacctctgacacccgagcagttccggtacaacaacgaggatgtgatccacgctccttacctggctcaccaaggatggtacgacatcaccaaggtgttcgacggcaaggacaacctgctgtgtggcgctgctaccgccggcaatatgctgcactggtggttcgaccagaacaagaccgagatcgaggcctacctgagcaagcaccccgagaagcagaagatcatcttcaacaatcaagagctgttcgacctgaaggccgccatcgacaccaaggactcccagaccaacagccagctgttcaactacttccgcgacaaggcctttcctaacctgtctgctagacagctgggcgtgatgcctgacctggtgctggacatgttcatcaacggctactacctgaacgtgttcaagacccagtccaccgacgtgaaccggccttaccaggacaaggataagagaggcggcatcttcgacgccgtgttcaccagaggcgatcagaccacactgctgaccgccagacacgatctgaagaacaagggcctgaacgacatctccaccatcatcaagcaagagctgaccgagggcagagccctggctctgtctcacacctacgccaacgtgtccatcagccacgtgatcaacctgtggggcgctgactttaacgccgagggcaatctggaagccatctacgtgaccgactctgacgccaacgcctccatcggcatgaagaaatacttcgtgggcatcaacgctcacggccatgtggccatctccgccaagaagatcgagggcgagaatatcggcgctcaggtgctgggcctgttcaccctgagttccggcaaggatatctggcagaagctgtcc

SEQ ID NO: 3 - protein, 315 aa, Streptococcus equi
DDYQRNAAEVYAKEVPHQITSVWTKGVTPLTPEQFRYNNEDVIHAPYLAHQGWYDITKVFDGKDNLLCGAATAGNMLHWWFDQNKTEIEAYLSKHPEKQKIIFNNQELFDLKAAIDTKDSQTNSQLFNYFRDKAFPNLSARQLGVMPDLVLDMFINGYYLNVFKTQSTDVNRPYQDKDKRGGIFDAVFTRGDQTTLLTARHDLKNKGLNDISTIIKQELTEGRALALSHTYANVSISHVINLWGADFNAEGNLEAIYVTDSDANASIGMKKYFVGINAHGHVAISAKKIEGENIGAQVLGLFTLSSGKDIWQKLS

SEQ ID NO: 4 - DNA, 945 bp, Streptococcus equi
  source 1..945: mol_type = other DNA
gacgactaccagagaaacgccgccgaggtgtacgccaaagaggtgccacatcagatcacctccgtgtggaccaagggcgtgacacctctgacacccgagcagttccggtacaacaacgaggatgtgatccacgctccttacctggctcaccaaggatggtacgacatcaccaaggtgttcgacggcaaggacaacctgctgtgtggcgctgctaccgccggcaatatgctgcactggtggttcgaccagaacaaagaggaaatcgaggcctacctgagcaagcaccccgagaagcagaagatcatcttcaacaatcaagagctgttcgacctgaaggccgccatcgacaccaaggactcccagaccaacagccagctgttcaactacttccgcgacaaggcctttcctggcctgtccgctagacagctgggagtgatgcctgacctggtgctggacatgttcatcaacggctactacctgaacgtgttcaagacccagtccaccgacgtgaaccggccttaccaggacaaggataagagaggcggcatcttcgacgccgtgttcaccagaggcgatcagaccacactgctgaccgccagacacgatctgaagaacaagggcctgaacgacatctccaccatcatcaagcaagagctgaccgagggcagagccctggctctgtctcacacctatgccaacgtgcggatctcccacgtgatcaacctgtggggcgctgactttaacgccgagggcaatctggaagccatctacgtgaccgactctgacgccgatgcctccatcggcatgaagaaatacttcgtgggcatcaacgcccacggccatgtggccatctctgccaagaagatcgagggcgagaatatcggcgctcaggtgctgggcctgttcaccctgagttccggcaaggatatctggcagaagctgtcc

SEQ ID NO: 5 - protein, 315 aa, Streptococcus equi
DDYQRNAAEVYAKEVPHQITSVWTKGVTPLTPEQFRYNNEDVIHAPYLAHQGWYDITKVFDGKDNLLCGAATAGNMLHWWFDQNKEEIEAYLSKHPEKQKIIFNNQELFDLKAAIDTKDSQTNSQLFNYFRDKAFPGLSARQLGVMPDLVLDMFINGYYLNVFKTQSTDVNRPYQDKDKRGGIFDAVFTRGDQTTLLTARHDLKNKGLNDISTIIKQELTEGRALALSHTYANVRISHVINLWGADFNAEGNLEAIYVTDSDADASIGMKKYFVGINAHGHVAISAKKIEGENIGAQVLGLFTLSSGKDIWQKLS

SEQ ID NO: 6 - DNA, 945 bp, Streptococcus equi
  source 1..945: mol_type = other DNA
gacgactaccagagaaacgccgccgaggtgtacgccaaagaggtgccacatcagatcacctccgtgtggaccaagggcgtgacacctctgacacccgagcagttccggtacaacaacgaggatgtgatccacgctccttacctggctcaccaaggatggtacgacatcaccaaggtgttcgacggcaaggacaacctgctgtgtggcgctgctaccgccggcaatatgctgcactggtggttcgaccagaacaaaacggaaatcgaggcctacctgagcaagcaccccgagaagcagaagatcatcttcaacaatcaagagctgttcgacctgaaggccgccatcgacaccaaggactcccagaccaacagccagctgttcaactacttccgcgacaaggcctttcctggcctgtccgctagacagctgggagtgatgcctgacctggtgctggacatgttcatcaacggctactacctgaacgtgttcaagacccagtccaccgacgtgaaccggccttaccaggacaaggataagagaggcggcatcttcgacgccgtgttcaccagaggcgatcagaccacactgctgaccgccagacacgatctgaagaacaagggcctgaacgacatctccaccatcatcaagcaagagctgaccgagggcagagccctggctctgtctcacacctatgccaacgtgcggatctcccacgtgatcaacctgtggggcgctgactttaacgccgagggcaatctggaagccatctacgtgaccgactctgacgccgatgcctccatcggcatgaagaaatacttcgtgggcatcaacgcccacggccatgtggccatctctgccaagaagatcgagggcgagaatatcggcgctcaggtgctgggcctgttcaccctgagttccggcaaggatatctggcagaagctgtcc

SEQ ID NO: 7 - protein, 315 aa, Streptococcus equi
DDYQRNAAEVYAKEVPHQITSVWTKGVTPLTPEQFRYNNEDVIHAPYLAHQGWYDITKVFDGKDNLLCGAATAGNMLHWWFDQNKTEIEAYLSKHPEKQKIIFNNQELFDLKAAIDTKDSQTNSQLFNYFRDKAFPGLSARQLGVMPDLVLDMFINGYYLNVFKTQSTDVNRPYQDKDKRGGIFDAVFTRGDQTTLLTARHDLKNKGLNDISTIIKQELTEGRALALSHTYANVRISHVINLWGADFNAEGNLEAIYVTDSDADASIGMKKYFVGINAHGHVAISAKKIEGENIGAQVLGLFTLSSGKDIWQKLS

SEQ ID NO: 8 - DNA, 945 bp, Streptococcus equi
  source 1..945: mol_type = other DNA
gacgactaccagagaaacgccgccgaggtgtacgccaaagaggtgccacatcagatcacctccgtgtggaccaagggcgtgacacctctgacacccgagcagttccggtacaacaacgaggatgtgatccacgctccttacctggctcaccaaggatggtacgacatcaccaaggtgttcgacggcaaggacaacctgctgtgtggcgctgctaccgccggcaatatgctgcactggtggttcgaccagaacaaagaggaaatcgaggcctacctgagcaagcaccccgagaagcagaagatcatcttcaacaatcaagagctgttcgacctgaaggccgccatcgacaccaaggactcccagaccaacagccagctgttcaactacttccgcgacaaggcctttcctaacctgtccgctagacagctgggagtgatgcctgacctggtgctggacatgttcatcaacggctactacctgaacgtgttcaagacccagtccaccgacgtgaaccggccttaccaggacaaggataagagaggcggcatcttcgacgccgtgttcaccagaggcgatcagaccacactgctgaccgccagacacgatctgaagaacaagggcctgaacgacatctccaccatcatcaagcaagagctgaccgagggcagagccctggctctgtctcacacctatgccaacgtgcggatctcccacgtgatcaacctgtggggcgctgactttaacgccgagggcaatctggaagccatctacgtgaccgactctgacgccgatgcctccatcggcatgaagaaatacttcgtgggcatcaacgcccacggccatgtggccatctctgccaagaagatcgagggcgagaatatcggcgctcaggtgctgggcctgttcaccctgagttccggcaaggatatctggcagaagctgtcc

SEQ ID NO: 9 - protein, 315 aa, Streptococcus equi
DDYQRNAAEVYAKEVPHQITSVWTKGVTPLTPEQFRYNNEDVIHAPYLAHQGWYDITKVFDGKDNLLCGAATAGNMLHWWFDQNKEEIEAYLSKHPEKQKIIFNNQELFDLKAAIDTKDSQTNSQLFNYFRDKAFPNLSARQLGVMPDLVLDMFINGYYLNVFKTQSTDVNRPYQDKDKRGGIFDAVFTRGDQTTLLTARHDLKNKGLNDISTIIKQELTEGRALALSHTYANVRISHVINLWGADFNAEGNLEAIYVTDSDADASIGMKKYFVGINAHGHVAISAKKIEGENIGAQVLGLFTLSSGKDIWQKLS

SEQ ID NO: 10 - DNA, 945 bp, Streptococcus equi
  source 1..945: mol_type = other DNA
gacgactaccagagaaacgccgccgaggtgtacgccaaagaggtgccacatcagatcacctccgtgtggaccaagggcgtgacacctctgacacccgagcagttccggtacaacaacgaggatgtgatccacgctccttacctggctcaccaaggatggtacgacatcaccaaggtgttcgacggcaaggacaacctgctgtgtggcgctgctaccgccggcaatatgctgcactggtggttcgaccagaacaaagaggaaatcgaggcctacctgagcaagcaccccgagaagcagaagatcatcttcaacaatcaagagctgttcgacctgaaggccgccatcgacaccaaggactcccagaccaacagccagctgttcaactacttccgcgacaaggcctttcctggcctgtccgctagacagctgggagtgatgcctgacctggtgctggacatgttcatcaacggctactacctgaacgtgttcaagacccagtccaccgacgtgaaccggccttaccaggacaaggataagagaggcggcatcttcgacgccgtgttcaccagaggcgatcagaccacactgctgaccgccagacacgatctgaagaacaagggcctgaacgacatctccaccatcatcaagcaagagctgaccgagggcagagccctggctctgtctcacacctatgccaacgtgtcgatctcccacgtgatcaacctgtggggcgctgactttaacgccgagggcaatctggaagccatctacgtgaccgactctgacgccgatgcctccatcggcatgaagaaatacttcgtgggcatcaacgcccacggccatgtggccatctctgccaagaagatcgagggcgagaatatcggcgctcaggtgctgggcctgttcaccctgagttccggcaaggatatctggcagaagctgtcc

SEQ ID NO: 11 - protein, 315 aa, Streptococcus equi
DDYQRNAAEVYAKEVPHQITSVWTKGVTPLTPEQFRYNNEDVIHAPYLAHQGWYDITKVFDGKDNLLCGAATAGNMLHWWFDQNKEEIEAYLSKHPEKQKIIFNNQELFDLKAAIDTKDSQTNSQLFNYFRDKAFPGLSARQLGVMPDLVLDMFINGYYLNVFKTQSTDVNRPYQDKDKRGGIFDAVFTRGDQTTLLTARHDLKNKGLNDISTIIKQELTEGRALALSHTYANVSISHVINLWGADFNAEGNLEAIYVTDSDADASIGMKKYFVGINAHGHVAISAKKIEGENIGAQVLGLFTLSSGKDIWQKLS

SEQ ID NO: 12 - DNA, 945 bp, Streptococcus equi
  source 1..945: mol_type = other DNA
gacgactaccagagaaacgccgccgaggtgtacgccaaagaggtgccacatcagatcacctccgtgtggaccaagggcgtgacacctctgacacccgagcagttccggtacaacaacgaggatgtgatccacgctccttacctggctcaccaaggatggtacgacatcaccaaggtgttcgacggcaaggacaacctgctgtgtggcgctgctaccgccggcaatatgctgcactggtggttcgaccagaacaaagaggaaatcgaggcctacctgagcaagcaccccgagaagcagaagatcatcttcaacaatcaagagctgttcgacctgaaggccgccatcgacaccaaggactcccagaccaacagccagctgttcaactacttccgcgacaaggcctttcctggcctgtccgctagacagctgggagtgatgcctgacctggtgctggacatgttcatcaacggctactacctgaacgtgttcaagacccagtccaccgacgtgaaccggccttaccaggacaaggataagagaggcggcatcttcgacgccgtgttcaccagaggcgatcagaccacactgctgaccgccagacacgatctgaagaacaagggcctgaacgacatctccaccatcatcaagcaagagctgaccgagggcagagccctggctctgtctcacacctatgccaacgtgcggatctcccacgtgatcaacctgtggggcgctgactttaacgccgagggcaatctggaagccatctacgtgaccgactctgacgccaatgcctccatcggcatgaagaaatacttcgtgggcatcaacgcccacggccatgtggccatctctgccaagaagatcgagggcgagaatatcggcgctcaggtgctgggcctgttcaccctgagttccggcaaggatatctggcagaagctgtcc

SEQ ID NO: 13 - protein, 315 aa, Streptococcus equi
DDYQRNAAEVYAKEVPHQITSVWTKGVTPLTPEQFRYNNEDVIHAPYLAHQGWYDITKVFDGKDNLLCGAATAGNMLHWWFDQNKEEIEAYLSKHPEKQKIIFNNQELFDLKAAIDTKDSQTNSQLFNYFRDKAFPGLSARQLGVMPDLVLDMFINGYYLNVFKTQSTDVNRPYQDKDKRGGIFDAVFTRGDQTTLLTARHDLKNKGLNDISTIIKQELTEGRALALSHTYANVRISHVINLWGADFNAEGNLEAIYVTDSDANASIGMKKYFVGINAHGHVAISAKKIEGENIGAQVLGLFTLSSGKDIWQKLS

SEQ ID NO: 14 - protein, 541 aa, synthetic construct
DDYQRNAAEVYAKEVPHQITSVWTKGVTPLTPEQFRYNNEDVIHAPYLAHQGWYDITKVFDGKDNLLCGAATAGNMLHWWFDQNKEEIEAYLSKHPEKQKIIFNNQELFDLKAAIDTKDSQTNSQLFNYFRDKAFPGLSARQLGVMPDLVLDMFINGYYLNVFKTQSTDVNRPYQDKDKRGGIFDAVFTRGDQTTLLTARHDLKNKGLNDISTIIKQELTEGRALALSHTYANVRISHVINLWGADFNAEGNLEAIYVTDSDADASIGMKKYFVGINAHGHVAISAKKIEGENIGAQVLGLFTLSSGKDIWQKLSDKTHTCPPCPAPNAEGGPSVFLFPPKPKDTLMASRTPEVTCVVVDVSHEDPEVKFNWYVDGVEVHNAKTKPREQYNSTYRVVSVLTVLHQDWLNGKEYKCKVSNKALPAPIEKTISKAKGQPREPQVYTLPPSRDELTKNQVSLTCLVKGFYPSDIAVEWESNGQPENNYKTTPPVLDSDGSFFLYSKLTVDKSRWQQGNVFSCSVMHEALHNHYTQKSLSLSPGK

SEQ ID NO: 15 - protein, 541 aa, synthetic construct
DDYQRNAAEVYAKEVPHQITSVWTKGVTPLTPEQFRYNNEDVIHAPYLAHQGWYDITKVFDGKDNLLCGAATAGNMLHWWFDQNKEEIEAYLSKHPEKQKIIFNNQELFDLKAAIDTKDSQTNSQLFNYFRDKAFPGLSARQLGVMPDLVLDMFINGYYLNVFKTQSTDVNRPYQDKDKRGGIFDAVFTRGDQTTLLTARHDLKNKGLNDISTIIKQELTEGRALALSHTYANVRISHVINLWGADFNAEGNLEAIYVTDSDADASIGMKKYFVGINAHGHVAISAKKIEGENIGAQVLGLFTLSSGKDIWQKLSDKTHTCHKCPAPNAEGGPSVFLFPPKPKDTLMASRTPEVTCVVVDVSHEDPEVKFNWYVDGVEVHNAKTKPREQYNSTYRVVSVLTVLHQDWLNGKEYKCKVSNKALPAPIEKTISKAKGQPREPQVYTLPPSRDELTKNQVSLTCLVKGFYPSDIAVEWESNGQPENNYKTTPPVLDSDGSFFLYSKLTVDKSRWQQGNVFSCSVMHEALHNHYTQKSLSLSPGK

SEQ ID NO: 16 - protein, 541 aa, synthetic construct
DDYQRNAAEVYAKEVPHQITSVWTKGVTPLTPEQFRYNNEDVIHAPYLAHQGWYDITKVFDGKDNLLCGAATAGNMLHWWFDQNKEEIEAYLSKHPEKQKIIFNNQELFDLKAAIDTKDSQTNSQLFNYFRDKAFPGLSARQLGVMPDLVLDMFINGYYLNVFKTQSTDVNRPYQDKDKRGGIFDAVFTRGDQTTLLTARHDLKNKGLNDISTIIKQELTEGRALALSHTYANVRISHVINLWGADFNAEGNLEAIYVTDSDADASIGMKKYFVGINAHGHVAISAKKIEGENIGAQVLGLFTLSSGKDIWQKLSDKTHTCPPCPAPEAEEVPSVFLFPPKPKDTLMASRTPEVTCVVVDVSHEDPEVKFNWYVDGVEVHNAKTKPREQYNSTYRVVSVLTVLHQDWLNGKEYKCKVSNKALPAPIEKTISKAKGQPREPQVYTLPPSRDELTKNQVSLTCLVKGFYPSDIAVEWESNGQPENNYKTTPPVLDSDGSFFLYSKLTVDKSRWQQGNVFSCSVMHEALHNHYTQKSLSLSPGK

SEQ ID NO: 17 - protein, 541 aa, synthetic construct
DDYQRNAAEVYAKEVPHQITSVWTKGVTPLTPEQFRYNNEDVIHAPYLAHQGWYDITKVFDGKDNLLCGAATAGNMLHWWFDQNKEEIEAYLSKHPEKQKIIFNNQELFDLKAAIDTKDSQTNSQLFNYFRDKAFPGLSARQLGVMPDLVLDMFINGYYLNVFKTQSTDVNRPYQDKDKRGGIFDAVFTRGDQTTLLTARHDLKNKGLNDISTIIKQELTEGRALALSHTYANVRISHVINLWGADFNAEGNLEAIYVTDSDADASIGMKKYFVGINAHGHVAISAKKIEGENIGAQVLGLFTLSSGKDIWQKLSDKTHTCHKCPAPNAEEVSSVFLFPPKPKDTLMASRTPEVTCVVVDVSHEDPEVKFNWYVDGVEVHNAKTKPREQYNSTYRVVSVLTVLHQDWLNGKEYKCKVSNKALPAPIEKTISKAKGQPREPQVYTLPPSRDELTKNQVSLTCLVKGFYPSDIAVEWESNGQPENNYKTTPPVLDSDGSFFLYSKLTVDKSRWQQGNVFSCSVMHEALHNHYTQKSLSLSPGK

SEQ ID NO: 18 - protein, 541 aa, synthetic construct
DDYQRNAAEVYAKEVPHQITSVWTKGVTPLTPEQFRYNNEDVIHAPYLAHQGWYDITKVFDGKDNLLCGAATAGNMLHWWFDQNKEEIEAYLSKHPEKQKIIFNNQELFDLKAAIDTKDSQTNSQLFNYFRDKAFPGLSARQLGVMPDLVLDMFINGYYLNVFKTQSTDVNRPYQDKDKRGGIFDAVFTRGDQTTLLTARHDLKNKGLNDISTIIKQELTEGRALALSHTYANVRISHVINLWGADFNAEGNLEAIYVTDSDADASIGMKKYFVGINAHGHVAISAKKIEGENIGAQVLGLFTLSSGKDIWQKLSDKTHTCPPCPAPEAEGGPSVFLFPPKPKDTLMASRTPEVTCVVVDVSHEDPEVKFNWYVDGVEVHNAKTKPREQANSTYRVVSVLTVLHQDWLNGKEYKCKVSNKALPAPIEKTISKAKGQPREPQVYTLPPSRDELTKNQVSLTCLVKGFYPSDIAVEWESNGQPENNYKTTPPVLDSDGSFFLYSKLTVDKSRWQQGNVFSCSVMHEALHNHYTQKSLSLSPGK

SEQ ID NO: 19 - protein, 541 aa, synthetic construct
DDYQRNAAEVYAKEVPHQITSVWTKGVTPLTPEQFRYNNEDVIHAPYLAHQGWYDITKVFDGKDNLLCGAATAGNMLHWWFDQNKEEIEAYLSKHPEKQKIIFNNQELFDLKAAIDTKDSQTNSQLFNYFRDKAFPGLSARQLGVMPDLVLDMFINGYYLNVFKTQSTDVNRPYQDKDKRGGIFDAVFTRGDQTTLLTARHDLKNKGLNDISTIIKQELTEGRALALSHTYANVRISHVINLWGADFNAEGNLEAIYVTDSDADASIGMKKYFVGINAHGHVAISAKKIEGENIGAQVLGLFTLSSGKDIWQKLSDKTHTCPPCPAPEAEGGPSVFLFPPKPKDTLMASRTPEVTCVVVDVSHEDPEVKFNWYVDGVEVHNAKTKPREQYNSTYRVVSVLTVLHQDWLNGKEYKCKVSNKALPAPIEKTISKAKGQPREPQVYTLPPSRDELTKNQVSLTCLVKGFYPSDIAVEWESNGQPENNYKTTPPVLDSDGSFFLYSKLTVDKSRWQQGNVFSCSVMHEALHNHYTQKSLSLSPGK

SEQ ID NO: 20 - protein, 541 aa, synthetic construct
DDYQRNAAEVYAKEVPHQITSVWTKGVTPLTPEQFRYNNEDVIHAPYLAHQGWYDITKVFDGKDNLLCGAATAGNMLHWWFDQNKEEIEAYLSKHPEKQKIIFNNQELFDLKAAIDTKDSQTNSQLFNYFRDKAFPGLSARQLGVMPDLVLDMFINGYYLNVFKTQSTDVNRPYQDKDKRGGIFDAVFTRGDQTTLLTARHDLKNKGLNDISTIIKQELTEGRALALSHTYANVRISHVINLWGADFNAEGNLEAIYVTDSDADASIGMKKYFVGINAHGHVAISAKKIEGENIGAQVLGLFTLSSGKDIWQKLSDKTHTCPPCPAPNAAGGPSVFLFPPKPKDTLMASRTPEVTCVVVDVSHEDPEVKFNWYVDGVEVHNAKTKPREQANSTYRVVSVLTVLHQDWLNGKEYKCKVSNKALPAPIEKTISKAKGQPREPQVYTLPPSRDELTKNQVSLTCLVKGFYPSDIAVEWESNGQPENNYKTTPPVLDSDGSFFLYSKLTVDKSRWQQGNVFSCSVMHEALHNHYTQKSLSLSPGK

SEQ ID NO: 21 - protein, 541 aa, synthetic construct
DDYQRNAAEVYAKEVPHQITSVWTKGVTPLTPEQFRYNNEDVIHAPYLAHQGWYDITKVFDGKDNLLCGAATAGNMLHWWFDQNKEEIEAYLSKHPEKQKIIFNNQELFDLKAAIDTKDSQTNSQLFNYFRDKAFPGLSARQLGVMPDLVLDMFINGYYLNVFKTQSTDVNRPYQDKDKRGGIFDAVFTRGDQTTLLTARHDLKNKGLNDISTIIKQELTEGRALALSHTYANVRISHVINLWGADFNAEGNLEAIYVTDSDADASIGMKKYFVGINAHGHVAISAKKIEGENIGAQVLGLFTLSSGKDIWQKLSDKTHTCPPCPAPEAEEVPSVFLFPPKPKDTLMASRTPEVTCVVVDVSHEDPEVKFNWYVDGVEVHNAKTKPREQANSTYRVVSVLTVLHQDWLNGKEYKCKVSNKALPAPIEKTISKAKGQPREPQVYTLPPSRDELTKNQVSLTCLVKGFYPSDIAVEWESNGQPENNYKTTPPVLDSDGSFFLYSKLTVDKSRWQQGNVFSCSVMHEALHNHYTQKSLSLSPGK

SEQ ID NO: 22 - protein, 541 aa, synthetic construct
DDYQRNAAEVYAKEVPHQITSVWTKGVTPLTPEQFRYNNEDVIHAPYLAHQGWYDITKVFDGKDNLLCGAATAGNMLHWWFDQNKEEIEAYLSKHPEKQKIIFNNQELFDLKAAIDTKDSQTNSQLFNYFRDKAFPGLSARQLGVMPDLVLDMFINGYYLNVFKTQSTDVNRPYQDKDKRGGIFDAVFTRGDQTTLLTARHDLKNKGLNDISTIIKQELTEGRALALSHTYANVRISHVINLWGADFNAEGNLEAIYVTDSDADASIGMKKYFVGINAHGHVAISAKKIEGENIGAQVLGLFTLSSGKDIWQKLSDKTHTCHKCPAPNAEEVSSVFLFPPKPKDTLMASRTPEVTCVVVDVSHEDPEVKFNWYVDGVEVHNAKTKPREQANSTYRVVSVLTVLHQDWLNGKEYKCKVSNKALPAPIEKTISKAKGQPREPQVYTLPPSRDELTKNQVSLTCLVKGFYPSDIAVEWESNGQPENNYKTTPPVLDSDGSFFLYSKLTVDKSRWQQGNVFSCSVMHEALHNHYTQKSLSLSPGK

SEQ ID NO: 23 - protein, 541 aa, synthetic construct
DDYQRNAAEVYAKEVPHQITSVWTKGVTPLTPEQFRYNNEDVIHAPYLAHQGWYDITKVFDGKDNLLCGAATAGNMLHWWFDQNKEEIEAYLSKHPEKQKIIFNNQELFDLKAAIDTKDSQTNSQLFNYFRDKAFPGLSARQLGVMPDLVLDMFINGYYLNVFKTQSTDVNRPYQDKDKRGGIFDAVFTRGDQTTLLTARHDLKNKGLNDISTIIKQELTEGRALALSHTYANVRISHVINLWGADFNAEGNLEAIYVTDSDADASIGMKKYFVGINAHGHVAISAKKIEGENIGAQVLGLFTLSSGKDIWQKLSDKTHTCPPCPAPEAEEVPSVFLFPPKPKDTLMASRTPEVTCVVVDVSHEDPEVKFNWYVDGVEVHNAKTKPREQYNSTYRVVSVLTVLHQDWLNGKEYKCKVSNKALPAPIEKTISKAKGQPREPQVYTLPPSRDELTKNQVSLSCAVKGFYPSDIAVEWESNGQPENNYKTTPPVLDSDGSFFLVSKLTVDKSRWQQGNVFSCSVMHEALHNHYTQKSLSLSPGK

SEQ ID NO: 24 - protein, 221 aa, synthetic construct
CPPCPAPEAEEVPSVFLFPPKPKDTLMASRTPEVTCVVVDVSHEDPEVKFNWYVDGVEVHNAKTKPREQYNSTYRVVSVLTVLHQDWLNGKEYKCKVSNKALPAPIEKTISKAKGQPREPQVYTLPPSRDELTKNQVSLWCLVKGFYPSDIAVEWESNGQPENNYKTTPPVLDSDGSFFLYSKLTVDKSRWQQGNVFSCSVMHEALHNHYTQKSLSLSPGK

SEQ ID NO: 25 - DNA, 1623 bp, synthetic construct
  source 1..1623: mol_type = other DNA
gacgactaccagagaaatgccgccgaggtgtacgccaaagaggtgccacatcagatcacctccgtgtggaccaagggcgtgacacctctgacacccgagcagttccggtacaacaacgaggatgtgatccacgctccttacctggctcaccaaggatggtacgacatcaccaaggtgttcgacggcaaggacaacctgctgtgtggcgctgctaccgccggcaatatgctgcactggtggttcgaccagaacaaagaggaaatcgaggcctacctgagcaagcaccccgagaagcagaagatcatcttcaacaatcaagagctgttcgacctgaaggccgccatcgacaccaaggactcccagaccaacagccagctgttcaactacttccgcgacaaggcctttcctggcctgtccgctagacagctgggagtgatgcctgacctggtgctggacatgttcatcaacggctactacctgaacgtgttcaagacccagtccaccgacgtgaaccggccttaccaggacaaggataagagaggcggcatcttcgacgccgtgttcaccagaggcgatcagaccacactgctgaccgccagacacgatctgaagaacaagggcctgaacgacatctccaccatcatcaagcaagagctgaccgagggcagagccctggctctgtctcacacctatgccaacgtgcggatctcccacgtgatcaacctgtggggcgctgactttaacgccgagggcaatctggaagccatctacgtgaccgactctgacgccgatgcctccatcggcatgaagaaatacttcgtgggcatcaacgcccacggccatgtggccatctctgccaagaagatcgagggcgagaatatcggcgctcaggtgctgggcctgttcaccctgagttccggcaaggatatctggcagaagctgtccgacaagacccacacctgtcctccatgtcctgctcctaatgctgaaggcggcccttccgtgtttctgttccctccaaagcctaaggacaccctgatggcctctcggacccctgaagtgacatgcgtggtggtggatgtgtcccacgaggacccagaagtgaagttcaattggtacgtggacggcgtggaagtgcacaacgccaagaccaagcctagagagcagtacaactccacctacagagtggtgtccgtgctgaccgtgctgcaccaggattggctgaacggcaaagagtacaagtgcaaggtgtccaacaaggccctgcctgctccaatcgaaaagaccatctccaaggccaagggccagcctagggaaccccaggtttacaccttgcctccatctcgggacgagctgaccaagaaccaggtgtccctgacctgtctcgtgaagggcttctacccctccgatatcgccgtggaatgggagtctaatggccagccagagaacaactacaagacaacccctcctgtgctggactccgacggctcattctttctgtactccaagctgacagtggacaagtccagatggcagcagggcaacgtgttctcctgcagcgtgatgcacgaggccctgcacaatcactacacacagaagtccctgtctctgtcccctggcaag

SEQ ID NO: 26 - DNA, 1623 bp, synthetic construct
  source 1..1623: mol_type = other DNA
gacgactaccagagaaatgccgccgaggtgtacgccaaagaggtgccacatcagatcacctccgtgtggaccaagggcgtgacacctctgacacccgagcagttccggtacaacaacgaggatgtgatccacgctccttacctggctcaccaaggatggtacgacatcaccaaggtgttcgacggcaaggacaacctgctgtgtggcgctgctaccgccggcaatatgctgcactggtggttcgaccagaacaaagaggaaatcgaggcctacctgagcaagcaccccgagaagcagaagatcatcttcaacaatcaagagctgttcgacctgaaggccgccatcgacaccaaggactcccagaccaacagccagctgttcaactacttccgcgacaaggcctttcctggcctgtccgctagacagctgggagtgatgcctgacctggtgctggacatgttcatcaacggctactacctgaacgtgttcaagacccagtccaccgacgtgaaccggccttaccaggacaaggataagagaggcggcatcttcgacgccgtgttcaccagaggcgatcagaccacactgctgaccgccagacacgatctgaagaacaagggcctgaacgacatctccaccatcatcaagcaagagctgaccgagggcagagccctggctctgtctcacacctatgccaacgtgcggatctcccacgtgatcaacctgtggggcgctgactttaacgccgagggcaatctggaagccatctacgtgaccgactctgacgccgatgcctccatcggcatgaagaaatacttcgtgggcatcaacgcccacggccatgtggccatctctgccaagaagatcgagggcgagaatatcggcgctcaggtgctgggcctgttcaccctgagttccggcaaggatatctggcagaagctgtccgacaagacccacacctgtcacaagtgccctgctcctaatgctgaaggcggcccttccgtgtttctgttccctccaaagcctaaggacaccctgatggcctctcggacccctgaagtgacatgcgtggtggtggatgtgtcccacgaggacccagaagtgaagttcaattggtacgtggacggcgtggaagtgcacaacgccaagaccaagcctagagagcagtacaactccacctacagagtggtgtccgtgctgaccgtgctgcaccaggattggctgaacggcaaagagtacaagtgcaaggtgtccaacaaggccctgcctgctccaatcgaaaagaccatctccaaggccaagggccagcctagggaaccccaggtttacaccttgcctccatctcgggacgagctgaccaagaaccaggtgtccctgacctgtctcgtgaagggcttctacccctccgatatcgccgtggaatgggagtctaatggccagccagagaacaactacaagacaacccctcctgtgctggactccgacggctcattctttctgtactccaagctgacagtggacaagtccagatggcagcagggcaacgtgttctcctgcagcgtgatgcacgaggccctgcacaatcactacacacagaagtccctgtctctgtcccctggcaag

SEQ ID NO: 27 - DNA, 1623 bp, synthetic construct
  source 1..1623: mol_type = other DNA
gacgactaccagagaaatgccgccgaggtgtacgccaaagaggtgccacatcagatcacctccgtgtggaccaagggcgtgacacctctgacacccgagcagttccggtacaacaacgaggatgtgatccacgctccttacctggctcaccaaggatggtacgacatcaccaaggtgttcgacggcaaggacaacctgctgtgtggcgctgctaccgccggcaatatgctgcactggtggttcgaccagaacaaagaggaaatcgaggcctacctgagcaagcaccccgagaagcagaagatcatcttcaacaatcaagagctgttcgacctgaaggccgccatcgacaccaaggactcccagaccaacagccagctgttcaactacttccgcgacaaggcctttcctggcctgtccgctagacagctgggagtgatgcctgacctggtgctggacatgttcatcaacggctactacctgaacgtgttcaagacccagtccaccgacgtgaaccggccttaccaggacaaggataagagaggcggcatcttcgacgccgtgttcaccagaggcgatcagaccacactgctgaccgccagacacgatctgaagaacaagggcctgaacgacatctccaccatcatcaagcaagagctgaccgagggcagagccctggctctgtctcacacctatgccaacgtgcggatctcccacgtgatcaacctgtggggcgctgactttaacgccgagggcaatctggaagccatctacgtgaccgactctgacgccgatgcctccatcggcatgaagaaatacttcgtgggcatcaacgcccacggccatgtggccatctctgccaagaagatcgagggcgagaatatcggcgctcaggtgctgggcctgttcaccctgagttccggcaaggatatctggcagaagctgtccgacaagacccacacctgtcctccatgtcctgctccagaggctgaagaggtgccctccgtgtttctgttccctccaaagcctaaggacaccctgatggcctctcggacccctgaagtgacatgcgtggtggtggatgtgtcccacgaggacccagaagtgaagttcaattggtacgtggacggcgtggaagtgcacaacgccaagaccaagcctagagagcagtacaactccacctacagagtggtgtccgtgctgaccgtgctgcaccaggattggctgaacggcaaagagtacaagtgcaaggtgtccaacaaggccctgcctgctcctatcgaaaagaccatctccaaggccaagggccagcctagggaaccccaggtttacaccttgcctccatctcgggacgagctgaccaagaaccaggtgtccctgacctgtctcgtgaagggcttctacccctccgatatcgccgtggaatgggagtctaatggccagccagagaacaactacaagacaacccctcctgtgctggactccgacggctcattctttctgtactccaagctgacagtggacaagtccagatggcagcagggcaacgtgttctcctgcagcgtgatgcacgaggccctgcacaatcactacacacagaagtccctgtctctgtcccctggcaag

SEQ ID NO: 28 - DNA, 1623 bp, synthetic construct
  source 1..1623: mol_type = other DNA
gacgactaccagagaaatgccgccgaggtgtacgccaaagaggtgccacatcagatcacctccgtgtggaccaagggcgtgacacctctgacacccgagcagttccggtacaacaacgaggatgtgatccacgctccttacctggctcaccaaggatggtacgacatcaccaaggtgttcgacggcaaggacaacctgctgtgtggcgctgctaccgccggcaatatgctgcactggtggttcgaccagaacaaagaggaaatcgaggcctacctgagcaagcaccccgagaagcagaagatcatcttcaacaatcaagagctgttcgacctgaaggccgccatcgacaccaaggactcccagaccaacagccagctgttcaactacttccgcgacaaggcctttcctggcctgtccgctagacagctgggagtgatgcctgacctggtgctggacatgttcatcaacggctactacctgaacgtgttcaagacccagtccaccgacgtgaaccggccttaccaggacaaggataagagaggcggcatcttcgacgccgtgttcaccagaggcgatcagaccacactgctgaccgccagacacgatctgaagaacaagggcctgaacgacatctccaccatcatcaagcaagagctgaccgagggcagagccctggctctgtctcacacctatgccaacgtgcggatctcccacgtgatcaacctgtggggcgctgactttaacgccgagggcaatctggaagccatctacgtgaccgactctgacgccgatgcctccatcggcatgaagaaatacttcgtgggcatcaacgcccacggccatgtggccatctctgccaagaagatcgagggcgagaatatcggcgctcaggtgctgggcctgttcaccctgagttccggcaaggatatctggcagaagctgtccgacaagacccacacctgtcacaagtgccctgctcctaacgccgaagaggtgtcctccgtgtttctgttccctccaaagcctaaggacaccctgatggcctctcggacccctgaagtgacatgcgtggtggtggatgtgtcccacgaggacccagaagtgaagttcaattggtacgtggacggcgtggaagtgcacaacgccaagaccaagcctagagagcagtacaactccacctacagagtggtgtccgtgctgaccgtgctgcaccaggattggctgaacggcaaagagtacaagtgcaaggtgtccaacaaggccctgcctgctccaatcgaaaagaccatctccaaggccaagggccagcctagggaaccccaggtttacaccttgcctccatctcgggacgagctgaccaagaaccaggtgtccctgacctgtctcgtgaagggcttctacccctccgatatcgccgtggaatgggagtctaatggccagccagagaacaactacaagacaacccctcctgtgctggactccgacggctcattctttctgtactccaagctgacagtggacaagtccagatggcagcagggcaacgtgttctcctgcagcgtgatgcacgaggccctgcacaatcactacacacagaagtccctgtctctgtcccctggcaag

SEQ ID NO: 29 - DNA, 1623 bp, synthetic construct
  source 1..1623: mol_type = other DNA
gacgactaccagagaaatgccgccgaggtgtacgccaaagaggtgccacatcagatcacctccgtgtggaccaagggcgtgacacctctgacacccgagcagttccggtacaacaacgaggatgtgatccacgctccttacctggctcaccaaggatggtacgacatcaccaaggtgttcgacggcaaggacaacctgctgtgtggcgctgctaccgccggcaatatgctgcactggtggttcgaccagaacaaagaggaaatcgaggcctacctgagcaagcaccccgagaagcagaagatcatcttcaacaatcaagagctgttcgacctgaaggccgccatcgacaccaaggactcccagaccaacagccagctgttcaactacttccgcgacaaggcctttcctggcctgtccgctagacagctgggagtgatgcctgacctggtgctggacatgttcatcaacggctactacctgaacgtgttcaagacccagtccaccgacgtgaaccggccttaccaggacaaggataagagaggcggcatcttcgacgccgtgttcaccagaggcgatcagaccacactgctgaccgccagacacgatctgaagaacaagggcctgaacgacatctccaccatcatcaagcaagagctgaccgagggcagagccctggctctgtctcacacctatgccaacgtgcggatctcccacgtgatcaacctgtggggcgctgactttaacgccgagggcaatctggaagccatctacgtgaccgactctgacgccgatgcctccatcggcatgaagaaatacttcgtgggcatcaacgcccacggccatgtggccatctctgccaagaagatcgagggcgagaatatcggcgctcaggtgctgggcctgttcaccctgagttccggcaaggatatctggcagaagctgtccgacaagacccacacctgtcctccatgtcctgctccagaagctgaaggcggcccttccgtgtttctgttccctccaaagcctaaggacaccctgatggcctctcggacccctgaagtgacatgcgtggtggtggatgtgtcccacgaggatcccgaagtgaagttcaattggtacgtggacggcgtggaagtgcacaacgccaagaccaagcctagagagcaggccaactccacctacagagtggtgtctgtgctgaccgtgctgcaccaggattggctgaacggcaaagagtacaagtgcaaggtgtccaacaaggccctgcctgctcctatcgaaaagaccatctccaaggccaagggccagcctagggaaccccaggtttacaccttgccaccttctcgggacgagctgaccaagaaccaggtgtccctgacctgtctggtcaagggcttctacccctccgatatcgccgtggaatgggagtctaatggccagcctgagaacaactacaagacaacccctcctgtgctggactccgacggctcattctttctgtactccaagctgacagtggacaagtccagatggcagcagggcaacgtgttctcctgcagcgtgatgcacgaggccctgcacaatcactacacccagaagtccctgtctctgtcccctggcaag

SEQ ID NO: 30 - DNA, 1623 bp, synthetic construct
  source 1..1623: mol_type = other DNA
gacgactaccagagaaatgccgccgaggtgtacgccaaagaggtgccacatcagatcacctccgtgtggaccaagggcgtgacacctctgacacccgagcagttccggtacaacaacgaggatgtgatccacgctccttacctggctcaccaaggatggtacgacatcaccaaggtgttcgacggcaaggacaacctgctgtgtggcgctgctaccgccggcaatatgctgcactggtggttcgaccagaacaaagaggaaatcgaggcctacctgagcaagcaccccgagaagcagaagatcatcttcaacaatcaagagctgttcgacctgaaggccgccatcgacaccaaggactcccagaccaacagccagctgttcaactacttccgcgacaaggcctttcctggcctgtccgctagacagctgggagtgatgcctgacctggtgctggacatgttcatcaacggctactacctgaacgtgttcaagacccagtccaccgacgtgaaccggccttaccaggacaaggataagagaggcggcatcttcgacgccgtgttcaccagaggcgatcagaccacactgctgaccgccagacacgatctgaagaacaagggcctgaacgacatctccaccatcatcaagcaagagctgaccgagggcagagccctggctctgtctcacacctatgccaacgtgcggatctcccacgtgatcaacctgtggggcgctgactttaacgccgagggcaatctggaagccatctacgtgaccgactctgacgccgatgcctccatcggcatgaagaaatacttcgtgggcatcaacgcccacggccatgtggccatctctgccaagaagatcgagggcgagaatatcggcgctcaggtgctgggcctgttcaccctgagttccggcaaggatatctggcagaagctgtccgacaagacccacacctgtcctccatgtcctgctccagaagctgaaggcggcccttccgtgtttctgttccctccaaagcctaaggacaccctgatggcctctcggacccctgaagtgacatgcgtggtggtggatgtgtcccacgaggatcccgaagtgaagttcaattggtacgtggacggcgtggaagtgcacaacgccaagaccaagcctagagagcagtacaactccacctacagagtggtgtccgtgctgaccgtgctgcaccaggattggctgaacggcaaagagtacaagtgcaaggtgtccaacaaggccctgcctgctcctatcgaaaagaccatctccaaggccaagggccagcctagggaaccccaggtttacaccttgccaccttctcgggacgagctgaccaagaaccaggtgtccctgacctgtctggtcaagggcttctacccctccgatatcgccgtggaatgggagtctaatggccagcctgagaacaactacaagacaacccctcctgtgctggactccgacggctcattctttctgtactccaagctgacagtggacaagtccagatggcagcagggcaacgtgttctcctgcagcgtgatgcacgaggccctgcacaatcactacacccagaagtccctgtctctgtcccctggcaag

SEQ ID NO: 31 - DNA, 1623 bp, synthetic construct
  source 1..1623: mol_type = other DNA
gacgactaccagagaaatgccgccgaggtgtacgccaaagaggtgccacatcagatcacctccgtgtggaccaagggcgtgacacctctgacacccgagcagttccggtacaacaacgaggatgtgatccacgctccttacctggctcaccaaggatggtacgacatcaccaaggtgttcgacggcaaggacaacctgctgtgtggcgctgctaccgccggcaatatgctgcactggtggttcgaccagaacaaagaggaaatcgaggcctacctgagcaagcaccccgagaagcagaagatcatcttcaacaatcaagagctgttcgacctgaaggccgccatcgacaccaaggactcccagaccaacagccagctgttcaactacttccgcgacaaggcctttcctggcctgtccgctagacagctgggagtgatgcctgacctggtgctggacatgttcatcaacggctactacctgaacgtgttcaagacccagtccaccgacgtgaaccggccttaccaggacaaggataagagaggcggcatcttcgacgccgtgttcaccagaggcgatcagaccacactgctgaccgccagacacgatctgaagaacaagggcctgaacgacatctccaccatcatcaagcaagagctgaccgagggcagagccctggctctgtctcacacctatgccaacgtgcggatctcccacgtgatcaacctgtggggcgctgactttaacgccgagggcaatctggaagccatctacgtgaccgactctgacgccgatgcctccatcggcatgaagaaatacttcgtgggcatcaacgcccacggccatgtggccatctctgccaagaagatcgagggcgagaatatcggcgctcaggtgctgggcctgttcaccctgagttccggcaaggatatctggcagaagctgtccgacaagacccacacctgtcctccatgtcctgctcctaatgctgctggcggcccttccgtgtttctgttccctccaaagcctaaggacaccctgatggcctctcggacccctgaagtgacatgcgtggtggtggatgtgtcccacgaggatcccgaagtgaagttcaattggtacgtggacggcgtggaagtgcacaacgccaagaccaagcctagagagcaggccaactccacctacagagtggtgtctgtgctgaccgtgctgcaccaggattggctgaacggcaaagagtacaagtgcaaggtgtccaacaaggccctgcctgctccaatcgaaaagaccatctccaaggccaagggccagcctagggaaccccaggtttacaccttgccaccttctcgggacgagctgaccaagaaccaggtgtccctgacctgtctggtcaagggcttctacccctccgatatcgccgtggaatgggagtctaatggccagcctgagaacaactacaagacaacccctcctgtgctggactccgacggctcattctttctgtactccaagctgacagtggacaagtccagatggcagcagggcaacgtgttctcctgcagcgtgatgcacgaggccctgcacaatcactacacccagaagtccctgtctctgtcccctggcaag

SEQ ID NO: 32 - DNA, 1623 bp, synthetic construct
  source 1..1623: mol_type = other DNA
gacgactaccagagaaatgccgccgaggtgtacgccaaagaggtgccacatcagatcacctccgtgtggaccaagggcgtgacacctctgacacccgagcagttccggtacaacaacgaggatgtgatccacgctccttacctggctcaccaaggatggtacgacatcaccaaggtgttcgacggcaaggacaacctgctgtgtggcgctgctaccgccggcaatatgctgcactggtggttcgaccagaacaaagaggaaatcgaggcctacctgagcaagcaccccgagaagcagaagatcatcttcaacaatcaagagctgttcgacctgaaggccgccatcgacaccaaggactcccagaccaacagccagctgttcaactacttccgcgacaaggcctttcctggcctgtccgctagacagctgggagtgatgcctgacctggtgctggacatgttcatcaacggctactacctgaacgtgttcaagacccagtccaccgacgtgaaccggccttaccaggacaaggataagagaggcggcatcttcgacgccgtgttcaccagaggcgatcagaccacactgctgaccgccagacacgatctgaagaacaagggcctgaacgacatctccaccatcatcaagcaagagctgaccgagggcagagccctggctctgtctcacacctatgccaacgtgcggatctcccacgtgatcaacctgtggggcgctgactttaacgccgagggcaatctggaagccatctacgtgaccgactctgacgccgatgcctccatcggcatgaagaaatacttcgtgggcatcaacgcccacggccatgtggccatctctgccaagaagatcgagggcgagaatatcggcgctcaggtgctgggcctgttcaccctgagttccggcaaggatatctggcagaagctgtccgacaagacccacacctgtcctccatgtcctgctccagaggctgaagaggtgccctccgtgtttctgttccctccaaagcctaaggacaccctgatggcctctcggacccctgaagtgacatgcgtggtggtggatgtgtcccacgaggacccagaagtgaagttcaattggtacgtggacggcgtggaagtgcacaacgccaagaccaagcctagagagcaggccaactccacctacagagtggtgtccgtgctgaccgtgctgcaccaggattggctgaacggcaaagagtacaagtgcaaggtgtccaacaaggccctgcctgctcctatcgaaaagaccatctccaaggccaagggccagcctagggaaccccaggtttacaccttgcctccatctcgggacgagctgaccaagaaccaggtgtccctgacctgtctcgtgaagggcttctacccctccgatatcgccgtggaatgggagtctaatggccagccagagaacaactacaagacaacccctcctgtgctggactccgacggctcattctttctgtactccaagctgacagtggacaagtccagatggcagcagggcaacgtgttctcctgcagcgtgatgcacgaggccctgcacaatcactacacacagaagtccctgtctctgtcccctggcaag

SEQ ID NO: 33 - DNA, 1623 bp, synthetic construct
  source 1..1623: mol_type = other DNA
gacgactaccagagaaatgccgccgaggtgtacgccaaagaggtgccacatcagatcacctccgtgtggaccaagggcgtgacacctctgacacccgagcagttccggtacaacaacgaggatgtgatccacgctccttacctggctcaccaaggatggtacgacatcaccaaggtgttcgacggcaaggacaacctgctgtgtggcgctgctaccgccggcaatatgctgcactggtggttcgaccagaacaaagaggaaatcgaggcctacctgagcaagcaccccgagaagcagaagatcatcttcaacaatcaagagctgttcgacctgaaggccgccatcgacaccaaggactcccagaccaacagccagctgttcaactacttccgcgacaaggcctttcctggcctgtccgctagacagctgggagtgatgcctgacctggtgctggacatgttcatcaacggctactacctgaacgtgttcaagacccagtccaccgacgtgaaccggccttaccaggacaaggataagagaggcggcatcttcgacgccgtgttcaccagaggcgatcagaccacactgctgaccgccagacacgatctgaagaacaagggcctgaacgacatctccaccatcatcaagcaagagctgaccgagggcagagccctggctctgtctcacacctatgccaacgtgcggatctcccacgtgatcaacctgtggggcgctgactttaacgccgagggcaatctggaagccatctacgtgaccgactctgacgccgatgcctccatcggcatgaagaaatacttcgtgggcatcaacgcccacggccatgtggccatctctgccaagaagatcgagggcgagaatatcggcgctcaggtgctgggcctgttcaccctgagttccggcaaggatatctggcagaagctgtccgacaagacccacacctgtcacaagtgccctgctcctaacgccgaagaggtgtcctccgtgtttctgttccctccaaagcctaaggacaccctgatggcctctcggacccctgaagtgacatgcgtggtggtggatgtgtcccacgaggacccagaagtgaagttcaattggtacgtggacggcgtggaagtgcacaacgccaagaccaagcctagagagcaggccaactccacctacagagtggtgtccgtgctgaccgtgctgcaccaggattggctgaacggcaaagagtacaagtgcaaggtgtccaacaaggccctgcctgctccaatcgaaaagaccatctccaaggccaagggccagcctagggaaccccaggtttacaccttgcctccatctcgggacgagctgaccaagaaccaggtgtccctgacctgtctcgtgaagggcttctacccctccgatatcgccgtggaatgggagtctaatggccagccagagaacaactacaagacaacccctcctgtgctggactccgacggctcattctttctgtactccaagctgacagtggacaagtccagatggcagcagggcaacgtgttctcctgcagcgtgatgcacgaggccctgcacaatcactacacacagaagtccctgtctctgtcccctggcaag

SEQ ID NO: 34 - DNA, 1623 bp, synthetic construct
  source 1..1623: mol_type = other DNA
gacgactaccagagaaatgccgccgaggtgtacgccaaagaggtgccacatcagatcacctccgtgtggaccaagggcgtgacacctctgacacccgagcagttccggtacaacaacgaggatgtgatccacgctccttacctggctcaccaaggatggtacgacatcaccaaggtgttcgacggcaaggacaacctgctgtgtggcgctgctaccgccggcaatatgctgcactggtggttcgaccagaacaaagaggaaatcgaggcctacctgagcaagcaccccgagaagcagaagatcatcttcaacaatcaagagctgttcgacctgaaggccgccatcgacaccaaggactcccagaccaacagccagctgttcaactacttccgcgacaaggcctttcctggcctgtccgctagacagctgggagtgatgcctgacctggtgctggacatgttcatcaacggctactacctgaacgtgttcaagacccagtccaccgacgtgaaccggccttaccaggacaaggataagagaggcggcatcttcgacgccgtgttcaccagaggcgatcagaccacactgctgaccgccagacacgatctgaagaacaagggcctgaacgacatctccaccatcatcaagcaagagctgaccgagggcagagccctggctctgtctcacacctatgccaacgtgcggatctcccacgtgatcaacctgtggggcgctgactttaacgccgagggcaatctggaagccatctacgtgaccgactctgacgccgatgcctccatcggcatgaagaaatacttcgtgggcatcaacgcccacggccatgtggccatctctgccaagaagatcgagggcgagaatatcggcgctcaggtgctgggcctgttcaccctgagttccggcaaggatatctggcagaagctgtccgacaagacccacacctgtcctccatgtcctgctccagaggctgaagaggtcccctccgtgtttctgttccctccaaagcctaaggacaccctgatggcctctcggacccctgaagtgacatgcgtggtggtggatgtgtcccacgaggatcccgaagtgaagttcaattggtacgtggacggcgtggaagtgcacaacgccaagaccaagcctagagagcagtacaactccacctacagagtggtgtccgtgctgaccgtgctgcaccaggattggctgaacggcaaagagtacaagtgcaaggtgtccaacaaggccctgcctgctcctatcgaaaagaccatctccaaggccaagggccagcctagggaaccccaggtttacaccttgccaccttctcgggacgagctgaccaagaaccaggtgtccctgtcttgtgccgtgaagggcttctacccctccgatatcgctgtggaatgggagagcaatggccagcctgagaacaactacaagacaacccctcctgtgctggactccgacggctcattcttcctggtgtccaagctgacagtggacaagtccagatggcagcagggcaacgtgttctcctgcagcgtgatgcacgaggccctgcacaatcactacacccagaagtctctgtctctgtcccctggcaag

SEQ ID NO: 35 - DNA, 663 bp, synthetic construct
  source 1..663: mol_type = other DNA
tgtcctccatgtcctgcacctgaggctgaagaggtgccctccgtgtttctgttccctccaaagcctaaggacaccctgatggcctctcggacccctgaagtgacatgcgtggtggtggatgtgtcccacgaggatcccgaagtgaagttcaattggtacgtggacggcgtggaagtgcacaacgccaagaccaagcctagagagcagtacaactccacctacagagtggtgtccgtgctgaccgtgctgcaccaggattggctgaacggcaaagagtacaagtgcaaggtgtccaacaaggccctgcctgctcctatcgaaaagaccatctccaaggccaagggccagcctagggaaccccaggtttacaccttgcctccatctcgggacgagctgaccaagaaccaggtgtccctgtggtgtctggtcaagggcttctacccctccgatatcgccgtggaatgggagtctaatggccagcctgagaacaactacaagaccacacctcctgtgctggactccgacggctcattctttctgtactccaagctgacagtggacaagtccagatggcagcagggcaacgtgttctcctgcagcgtgatgcacgaggccctgcacaatcactacacccagaagtccctgtctctgtcccctggcaag